European Patent Application EP 4 624 496 A2, published October 1, 2025. Title: NOVEL NICOTINE-BINDING ANTIBODIES. Applicant: KALNIK, MATTHEW W. THISTED, THOMAS BELTRAMINELLI, NICOLA FALLOT, STEPHANIE BIESOVA, ZUZANA FULLER, STEVE LESAGE, MARK G. PENTEL, PAUL. Application PCT/US2018/046621. The sequence listing filed with the application follows.

SEQUENCE LISTING (40 sequences)

SEQ ID NO: 1 - protein, 447 aa, Artificial Sequence
  source: /note="Description of Artificial Sequence: Synthetic polypeptide"
QVRLQESGPGLVKPSGTLSLTCAVSGGSIYSSNWWTWVRQPPGKGLEWVGEIHIRGTTYYNPSLNSRVTISLDKSNNQVSLRLTSVTAADSAVYYCVSQEVGGPDLWGQGTLVTVSSASTKGPSVFPLAPSSKSTSGGTAALGCLVKDYFPEPVTVSWNSGALTSGVHTFPAVLQSSGLYSLSSVVTVPSSSLGTQTYICNVNHKPSNTKVDKKVEPKSCDKTHTCPPCPAPELLGGPSVFLFPPKPKDTLMISRTPEVTCVVVDVSHEDPEVKFNWYVDGVEVHNAKTKPREEQYNSTYRVVSVLTVLHQDWLNGKEYKCKVSNKALPAPIEKTISKAKGQPREPQVYTLPPSRDELTKNQVSLTCLVKGFYPSDIAVEWESNGQPENNYKTTPPVLDSDGSFFLYSKLTVDKSRWQQGNVFSCSVMHEALHNHYTQKSLSLSPGK

SEQ ID NO: 2 - protein, 216 aa, Artificial Sequence
  source: /note="Description of Artificial Sequence: Synthetic polypeptide"
NFMLTQPHSVSESPGKTVTISCTRSGGSIATYYVQWYQQRPGSAPTNVIYKYDQRPSGVPDRFSGSIDSSSNSASLTISGLKTEDEADYYCQSYDNNIQVFGGGTKLTVLGQPKAAPSVTLFPPSSEELQANKATLVCLISDFYPGAVTVAWKADGSPVKAGVETTKPSKQSNNKYAASSYLSLTPEQWKSHRSYSCQVTHEGSTVEKTVAPTECS

SEQ ID NO: 3 - protein, 453 aa, Artificial Sequence
  source: /note="Description of Artificial Sequence: Synthetic polypeptide"
QLQLQESGPGLVKPSETLSLICTVSGGSIRKNNEWWAWIRQAPGKGLEWIGSLSYTGRTVYNPSLKSRVTISTDTSETQFSLKVNSVTAADTAVYYCARLSPFVGAAWWFDPWGQGTLVTVSSASTKGPSVFPLAPSSKSTSGGTAALGCLVKDYFPEPVTVSWNSGALTSGVHTFPAVLQSSGLYSLSSVVTVPSSSLGTQTYICNVNHKPSNTKVDKKVEPKSCDKTHTCPPCPAPELLGGPSVFLFPPKPKDTLMISRTPEVTCVVVDVSHEDPEVKFNWYVDGVEVHNAKTKPREEQYNSTYRVVSVLTVLHQDWLNGKEYKCKVSNKALPAPIEKTISKAKGQPREPQVYTLPPSRDELTKNQVSLTCLVKGFYPSDIAVEWESNGQPENNYKTTPPVLDSDGSFFLYSKLTVDKSRWQQGNVFSCSVMHEALHNHYTQKSLSLSPGK

SEQ ID NO: 4 - protein, 217 aa, Artificial Sequence
  source: /note="Description of Artificial Sequence: Synthetic polypeptide"
EVVLTQSPGTLSLSPGERATLSCRASQSVSSRYLAWYQQKPGQAPRLLIYGASSRAIGTPDRFSGSGSGTDFTLTISRLEPEDFAVYYCQQYAYSPPAITFGGGTKVEIKRTVAAPSVFIFPPSDEQLKSGTASVVCLLNNFYPREAKVQWKVDNALQSGNSQESVTEQDSKDSTYSLSSTLTLSKADYEKHKVYACEVTHQGLSSPVTKSFNRGEC

SEQ ID NO: 5 - protein, 456 aa, Artificial Sequence
  source: /note="Description of Artificial Sequence: Synthetic polypeptide"
QLQLQESGPGLLKPSETLSLTCTVSGGSVTTSPDWWAWLRQSPGKGLEWIGSVSYTGRTVYNPSLKSRVTISLDTSKNHLSLRMTSATAADTAVFYCARLTPIDRFSADYYVLDIWGQGATVTVSSASTKGPSVFPLAPSSKSTSGGTAALGCLVKDYFPEPVTVSWNSGALTSGVHTFPAVLQSSGLYSLSSVVTVPSSSLGTQTYICNVNHKPSNTKVDKKVEPKSCDKTHTCPPCPAPELLGGPSVFLFPPKPKDTLMISRTPEVTCVVVDVSHEDPEVKFNWYVDGVEVHNAKTKPREEQYNSTYRVVSVLTVLHQDWLNGKEYKCKVSNKALPAPIEKTISKAKGQPREPQVYTLPPSRDELTKNQVSLTCLVKGFYPSDIAVEWESNGQPENNYKTTPPVLDSDGSFFLYSKLTVDKSRWQQGNVFSCSVMHEALHNHYTQKSLSLSPGK

SEQ ID NO: 6 - protein, 216 aa, Artificial Sequence
  source: /note="Description of Artificial Sequence: Synthetic polypeptide"
EIVMTQSPATLSVSPGERATLSCRASQSISSNLAWFQHKPGQAPRLLIFRSSTRATGTPPRFSGSGSGTEFTLTISSLQSEDFAVYFCQHYSYWPPLITFGQGTRLEIKRTVAAPSVFIFPPSDEQLKSGTASVVCLLNNFYPREAKVQWKVDNALQSGNSQESVTEQDSKDSTYSLSSTLTLSKADYEKHKVYACEVTHQGLSSPVTKSFNRGEC

SEQ ID NO: 7 - protein, 458 aa, Artificial Sequence
  source: /note="Description of Artificial Sequence: Synthetic polypeptide"
QLQLRESGPGLVKPSETLSLTCSVSGGSISSSSYYWGWIRQPPGKGLEWIGSIYYTGRTYYNPSLESRVTISVDTSKNQFSLKLSSVTAADTAVYYCAGLHYSWSALGGYYFYGMDVWGQGTTVTVSSASTKGPSVFPLAPSSKSTSGGTAALGCLVKDYFPEPVTVSWNSGALTSGVHTFPAVLQSSGLYSLSSVVTVPSSSLGTQTYICNVNHKPSNTKVDKKVEPKSCDKTHTCPPCPAPELLGGPSVFLFPPKPKDTLMISRTPEVTCVVVDVSHEDPEVKFNWYVDGVEVHNAKTKPREEQYNSTYRVVSVLTVLHQDWLNGKEYKCKVSNKALPAPIEKTISKAKGQPREPQVYTLPPSRDELTKNQVSLTCLVKGFYPSDIAVEWESNGQPENNYKTTPPVLDSDGSFFLYSKLTVDKSRWQQGNVFSCSVMHEALHNHYTQKSLSLSPGK

SEQ ID NO: 8 - protein, 217 aa, Artificial Sequence
  source: /note="Description of Artificial Sequence: Synthetic polypeptide"
EIVLTQSPGTLSLSPGERATLSCRASQSVSSRDLVWYQQKPGQAPRLLIYGASTRATGIPDRFSGSGSGTDFTLTISRLEPEDFAVYYCQKYGSSPPRITFGPGTKVDIKRTVAAPSVFIFPPSDEQLKSGTASVVCLLNNFYPREAKVQWKVDNALQSGNSQESVTEQDSKDSTYSLSSTLTLSKADYEKHKVYACEVTHQGLSSPVTKSFNRGEC

SEQ ID NO: 9 - protein, 452 aa, Artificial Sequence
  source: /note="Description of Artificial Sequence: Synthetic polypeptide"
QLQLQESGPGLVKPSETLSLTCSVSGGSISSSSYYWGWSRQSPGKGLEWIASIYYSGSTYYNPSLKSRVTIFIDTSKNQFSLKLSSVTAADTAIYYCARVGTSAMSRAFDMWGQGTMVTVSSASTKGPSVFPLAPSSKSTSGGTAALGCLVKDYFPEPVTVSWNSGALTSGVHTFPAVLQSSGLYSLSSVVTVPSSSLGTQTYICNVNHKPSNTKVDKKVEPKSCDKTHTCPPCPAPELLGGPSVFLFPPKPKDTLMISRTPEVTCVVVDVSHEDPEVKFNWYVDGVEVHNAKTKPREEQYNSTYRVVSVLTVLHQDWLNGKEYKCKVSNKALPAPIEKTISKAKGQPREPQVYTLPPSRDELTKNQVSLTCLVKGFYPSDIAVEWESNGQPENNYKTTPPVLDSDGSFFLYSKLTVDKSRWQQGNVFSCSVMHEALHNHYTQKSLSLSPGK

SEQ ID NO: 10 - protein, 219 aa, Artificial Sequence
  source: /note="Description of Artificial Sequence: Synthetic polypeptide"
DIVMTQSPLSLPVTPGEPASISCRSSQSLLQSNGYNYLDWYLQKPGQSPQLLIYLGSNRASGVPDRFSGSGSGTDFTLKISKVEAEDVGVYFCMQALQIPWTFGQGTKVEIKRTVAAPSVFIFPPSDEQLKSGTASVVCLLNNFYPREAKVQWKVDNALQSGNSQESVTEQDSKDSTYSLSSTLTLSKADYEKHKVYACEVTHQGLSSPVTKSFNRGEC

SEQ ID NO: 11 - protein, 453 aa, Artificial Sequence
  source: /note="Description of Artificial Sequence: Synthetic polypeptide"
QVQLQESGPGLVKPSETLSLTCTVSGGSISRRNDYWAWIRQSPGKDLEWIGTISFSGSTFYNPSLKSRVTISADTFNNHFSLRLDAVAAADTAVYYCARLSPFVGAAWWFDPWGPGTLVTVSSASTKGPSVFPLAPSSKSTSGGTAALGCLVKDYFPEPVTVSWNSGALTSGVHTFPAVLQSSGLYSLSSVVTVPSSSLGTQTYICNVNHKPSNTKVDKKVEPKSCDKTHTCPPCPAPELLGGPSVFLFPPKPKDTLMISRTPEVTCVVVDVSHEDPEVKFNWYVDGVEVHNAKTKPREEQYNSTYRVVSVLTVLHQDWLNGKEYKCKVSNKALPAPIEKTISKAKGQPREPQVYTLPPSRDELTKNQVSLTCLVKGFYPSDIAVEWESNGQPENNYKTTPPVLDSDGSFFLYSKLTVDKSRWQQGNVFSCSVMHEALHNHYTQKSLSLSPGK

SEQ ID NO: 12 - protein, 217 aa, Artificial Sequence
  source: /note="Description of Artificial Sequence: Synthetic polypeptide"
EIVLTQSPGTLSLSPGERATLSCRASQSLSSNYLGWYQQKPGQAPRLLIYGASNRATGIPDRFSGSGSGTDFTLTISRLEPEDFGVYYCQRYGRSPPAITFGGGTKVEIKRTVAAPSVFIFPPSDEQLKSGTASVVCLLNNFYPREAKVQWKVDNALQSGNSQESVTEQDSKDSTYSLSSTLTLSKADYEKHKVYACEVTHQGLSSPVTKSFNRGEC

SEQ ID NO: 13 - protein, 457 aa, Artificial Sequence
  source: /note="Description of Artificial Sequence: Synthetic polypeptide"
QLQLQESGPGLVKPSETLSLTCTASGGSITNNIDYWVWIRQPPGRGLEWIGTIYYSGSTFYNPSLKSRVTISVDTSNNQFSLNLNSMSAADTAVYYCARLRYYYDSNGYLPYWIDSWGQGTLVTVSSASTKGPSVFPLAPSSKSTSGGTAALGCLVKDYFPEPVTVSWNSGALTSGVHTFPAVLQSSGLYSLSSVVTVPSSSLGTQTYICNVNHKPSNTKVDKKVEPKSCDKTHTCPPCPAPELLGGPSVFLFPPKPKDTLMISRTPEVTCVVVDVSHEDPEVKFNWYVDGVEVHNAKTKPREEQYNSTYRVVSVLTVLHQDWLNGKEYKCKVSNKALPAPIEKTISKAKGQPREPQVYTLPPSRDELTKNQVSLTCLVKGFYPSDIAVEWESNGQPENNYKTTPPVLDSDGSFFLYSKLTVDKSRWQQGNVFSCSVMHEALHNHYTQKSLSLSPGK

SEQ ID NO: 14 - protein, 217 aa, Artificial Sequence
  source: /note="Description of Artificial Sequence: Synthetic polypeptide"
EIVLTQSPGTLSLSPGERATLSCRASQSISSSYLGWYQQKPGQAPRLLIYGASSRATGIPDRFSGSGSGTDFTLTISSLEPEDFAVYFCQLYRRSPPRLTFGGGTKVEIKRTVAAPSVFIFPPSDEQLKSGTASVVCLLNNFYPREAKVQWKVDNALQSGNSQESVTEQDSKDSTYSLSSTLTLSKADYEKHKVYACEVTHQGLSSPVTKSFNRGEC

SEQ ID NO: 15 - protein, 455 aa, Artificial Sequence
  source: /note="Description of Artificial Sequence: Synthetic polypeptide"
QLQLQESGPGLVKPSESLSLTCTVSGGSIISNDYYWAWIRQSPGKGLEWIGSINYRGSTFYSPSLNSRVTTSVDTSKNQFFLKLTSVTAADTAMYFCTRLHGRYRGVGRLAFDYWGQGTLVTVSSASTKGPSVFPLAPSSKSTSGGTAALGCLVKDYFPEPVTVSWNSGALTSGVHTFPAVLQSSGLYSLSSVVTVPSSSLGTQTYICNVNHKPSNTKVDKKVEPKSCDKTHTCPPCPAPELLGGPSVFLFPPKPKDTLMISRTPEVTCVVVDVSHEDPEVKFNWYVDGVEVHNAKTKPREEQYNSTYRVVSVLTVLHQDWLNGKEYKCKVSNKALPAPIEKTISKAKGQPREPQVYTLPPSRDELTKNQVSLTCLVKGFYPSDIAVEWESNGQPENNYKTTPPVLDSDGSFFLYSKLTVDKSRWQQGNVFSCSVMHEALHNHYTQKSLSLSPGK

SEQ ID NO: 16 - protein, 214 aa, Artificial Sequence
  source: /note="Description of Artificial Sequence: Synthetic polypeptide"
DIQMTQSPSTLSASVGDIVTITCRASQSIGDWLAWYQQKPGKAPKLLIYKASNLESGVPSRFSGSGSGTEFTLTISSLQSDDFATYYCQQYDSYSVTFGQGTKVEIKGTVAAPSVFIFPPSDEQLKSGTASVVCLLNNFYPREAKVQWKVDNALQSGNSQESVTEQDSKDSTYSLSSTLTLSKADYEKHKVYACEVTHQGLSSPVTKSFNRGEC

SEQ ID NO: 17 - protein, 456 aa, Artificial Sequence
  source: /note="Description of Artificial Sequence: Synthetic polypeptide"
QVQLQEAGPGLVKPSETLSLTCTVSGGSINTRNYYWGWVRQPPGKGLEWIASVYYTGSTFYDPSLRSRVTISIDTPRNQFSLRVSSVDAGDMGVYYCVRLDGGYNNGYYYYGMDVWGQGTSVTVSSASTKGPSVFPLAPSSKSTSGGTAALGCLVKDYFPEPVTVSWNSGALTSGVHTFPAVLQSSGLYSLSSVVTVPSSSLGTQTYICNVNHKPSNTKVDKKVEPKSCDKTHTCPPCPAPELLGGPSVFLFPPKPKDTLMISRTPEVTCVVVDVSHEDPEVKFNWYVDGVEVHNAKTKPREEQYNSTYRVVSVLTVLHQDWLNGKEYKCKVSNKALPAPIEKTISKAKGQPREPQVYTLPPSRDELTKNQVSLTCLVKGFYPSDIAVEWESNGQPENNYKTTPPVLDSDGSFFLYSKLTVDKSRWQQGNVFSCSVMHEALHNHYTQKSLSLSPGK

SEQ ID NO: 18 - protein, 214 aa, Artificial Sequence
  source: /note="Description of Artificial Sequence: Synthetic polypeptide"
GVQMTQSPSTLSASVGERVTVTCRASRPISNWLSWYQQKPGRAPKLLIYGTSTLESGVPSRFSGSGSGTEFTLTITNLQPDDFATYYCQEHNLYTITFGPGTKVEIKRTVAAPSVFIFPPSDEQLKSGTASVVCLLNNFYPREAKVQWKVDNALQSGNSQESVTEQDSKDSTYSLSSTLTLSKADYEKHKVYACEVTHQGLSSPVTKSFNRGEC

SEQ ID NO: 19 - protein, 457 aa, Artificial Sequence
  source: /note="Description of Artificial Sequence: Synthetic polypeptide"
QLQLQESGPGLVKPSETLSLSCAVSGASIRSNTYYWGWIRQPPGRGLEWIGSISHRGDAHYSPSLKSPVTISVDTSKNEFSLKATSVTAADTAVYYCVSLAYSFSWNTYYFYGMDVWGHGITVTVSSASTKGPSVFPLAPSSKSTSGGTAALGCLVKDYFPEPVTVSWNSGALTSGVHTFPAVLQSSGLYSLSSVVTVPSSSLGTQTYICNVNHKPSNTKVDKKVEPKSCDKTHTCPPCPAPELLGGPSVFLFPPKPKDTLMISRTPEVTCVVVDVSHEDPEVKFNWYVDGVEVHNAKTKPREEQYNSTYRVVSVLTVLHQDWLNGKEYKCKVSNKALPAPIEKTISKAKGQPREPQVYTLPPSRDELTKNQVSLTCLVKGFYPSDIAVEWESNGQPENNYKTTPPVLDSDGSFFLYSKLTVDKSRWQQGNVFSCSVMHEALHNHYTQKSLSLSPGK

SEQ ID NO: 20 - protein, 217 aa, Artificial Sequence
  source: /note="Description of Artificial Sequence: Synthetic polypeptide"
DIVLTQSPGTLSLSPGEGATLSCRASQSVNSGYLAWYQQKPGQPPRLLVFAASSRATGIADRFRGSGSGTDFTLTITRLEPEDFAVYYCQLYGHSPARITFGQGTRLETKRTVAAPSVFIFPPSDEQLKSGTASVVCLLNNFYPREAKVQWKVDNALQSGNSQESVTEQDSKDSTYSLSSTLTLSKADYEKHKVYACEVTHQGLSSPVTKSFNRGEC

SEQ ID NO: 21 - protein, 449 aa, Artificial Sequence
  source: /note="Description of Artificial Sequence: Synthetic polypeptide"
QLQLQESGPGLVKPSETLSLTCSVSGGSISSSSYYWGWSRQSPGKGLEWIASIYYSGSTYYNPSLKSRVTIFIDTSKNQFSLKLSSVTAADTAIYYCARVGTSAMSRAFDMWGQGTMVTVSSASTKGPSVFPLAPCSRSTSESTAALGCLVKDYFPEPVTVSWNSGALTSGVHTFPAVLQSSGLYSLSSVVTVPSSSLGTKTYTCNVDHKPSNTKVDKRVESKYGPPCPPCPAPEFLGGPSVFLFPPKPKDTLMISRTPEVTCVVVDVSQEDPEVQFNWYVDGVEVHNAKTKPREEQFNSTYRVVSVLTVLHQDWLNGKEYKCKVSNKGLPSSIEKTISKAKGQPREPQVYTLPPSQEEMTKNQVSLTCLVKGFYPSDIAVEWESNGQPENNYKTTPPVLDSDGSFFLYSRLTVDKSRWQEGNVFSCSVMHEALHNHYTQKSLSLSLGK

SEQ ID NO: 22 - protein, 219 aa, Artificial Sequence; identical to SEQ ID NO: 10
  source: /note="Description of Artificial Sequence: Synthetic polypeptide"

SEQ ID NO: 23 - protein, 453 aa, Artificial Sequence
  source: /note="Description of Artificial Sequence: Synthetic polypeptide"
QLQLQESGPGLLKPSETLSLTCTVSGGSVTTSPDWWAWLRQSPGKGLEWIGSVSYTGRTVYNPSLKSRVTISLDTSKNHLSLRMTSATAADTAVFYCARLTPIDRFSADYYVLDIWGQGATVTVSSASTKGPSVFPLAPCSRSTSESTAALGCLVKDYFPEPVTVSWNSGALTSGVHTFPAVLQSSGLYSLSSVVTVPSSSLGTKTYTCNVDHKPSNTKVDKRVESKYGPPCPPCPAPEFLGGPSVFLFPPKPKDTLMISRTPEVTCVVVDVSQEDPEVQFNWYVDGVEVHNAKTKPREEQFNSTYRVVSVLTVLHQDWLNGKEYKCKVSNKGLPSSIEKTISKAKGQPREPQVYTLPPSQEEMTKNQVSLTCLVKGFYPSDIAVEWESNGQPENNYKTTPPVLDSDGSFFLYSRLTVDKSRWQEGNVFSCSVMHEALHNHYTQKSLSLSLGK

SEQ ID NO: 24 - protein, 216 aa, Artificial Sequence; identical to SEQ ID NO: 6
  source: /note="Description of Artificial Sequence: Synthetic polypeptide"

SEQ ID NO: 25 - protein, 450 aa, Artificial Sequence
  source: /note="Description of Artificial Sequence: Synthetic polypeptide"
QLQLQESGPGLVKPSETLSLICTVSGGSIRKNNEWWAWIRQAPGKGLEWIGSLSYTGRTVYNPSLKSRVTISTDTSETQFSLKVNSVTAADTAVYYCARLSPFVGAAWWFDPWGQGTLVTVSSASTKGPSVFPLAPCSRSTSESTAALGCLVKDYFPEPVTVSWNSGALTSGVHTFPAVLQSSGLYSLSSVVTVPSSSLGTKTYTCNVDHKPSNTKVDKRVESKYGPPCPPCPAPEFLGGPSVFLFPPKPKDTLMISRTPEVTCVVVDVSQEDPEVQFNWYVDGVEVHNAKTKPREEQFNSTYRVVSVLTVLHQDWLNGKEYKCKVSNKGLPSSIEKTISKAKGQPREPQVYTLPPSQEEMTKNQVSLTCLVKGFYPSDIAVEWESNGQPENNYKTTPPVLDSDGSFFLYSRLTVDKSRWQEGNVFSCSVMHEALHNHYTQKSLSLSLGK

SEQ ID NO: 26 - protein, 217 aa, Artificial Sequence; identical to SEQ ID NO: 4
  source: /note="Description of Artificial Sequence: Synthetic polypeptide"

SEQ ID NO: 27 - protein, 444 aa, Artificial Sequence
  source: /note="Description of Artificial Sequence: Synthetic polypeptide"
QVRLQESGPGLVKPSGTLSLTCAVSGGSIYSSNWWTWVRQPPGKGLEWVGEIHIRGTTYYNPSLNSRVTISLDKSNNQVSLRLTSVTAADSAVYYCVSQEVGGPDLWGQGTLVTVSSASTKGPSVFPLAPCSRSTSESTAALGCLVKDYFPEPVTVSWNSGALTSGVHTFPAVLQSSGLYSLSSVVTVPSSSLGTKTYTCNVDHKPSNTKVDKRVESKYGPPCPPCPAPEFLGGPSVFLFPPKPKDTLMISRTPEVTCVVVDVSQEDPEVQFNWYVDGVEVHNAKTKPREEQFNSTYRVVSVLTVLHQDWLNGKEYKCKVSNKGLPSSIEKTISKAKGQPREPQVYTLPPSQEEMTKNQVSLTCLVKGFYPSDIAVEWESNGQPENNYKTTPPVLDSDGSFFLYSRLTVDKSRWQEGNVFSCSVMHEALHNHYTQKSLSLSLGK

SEQ ID NO: 28 - protein, 216 aa, Artificial Sequence; identical to SEQ ID NO: 2
  source: /note="Description of Artificial Sequence: Synthetic polypeptide"

SEQ ID NO: 29 - protein, 455 aa, Artificial Sequence
  source: /note="Description of Artificial Sequence: Synthetic polypeptide"
QLQLRESGPGLVKPSETLSLTCSVSGGSISSSSYYWGWIRQPPGKGLEWIGSIYYTGRTYYNPSLESRVTISVDTSKNQFSLKLSSVTAADTAVYYCAGLHYSWSALGGYYFYGMDVWGQGTTVTVSSASTKGPSVFPLAPCSRSTSESTAALGCLVKDYFPEPVTVSWNSGALTSGVHTFPAVLQSSGLYSLSSVVTVPSSSLGTKTYTCNVDHKPSNTKVDKRVESKYGPPCPPCPAPEFLGGPSVFLFPPKPKDTLMISRTPEVTCVVVDVSQEDPEVQFNWYVDGVEVHNAKTKPREEQFNSTYRVVSVLTVLHQDWLNGKEYKCKVSNKGLPSSIEKTISKAKGQPREPQVYTLPPSQEEMTKNQVSLTCLVKGFYPSDIAVEWESNGQPENNYKTTPPVLDSDGSFFLYSRLTVDKSRWQEGNVFSCSVMHEALHNHYTQKSLSLSLGK

SEQ ID NO: 30 - protein, 217 aa, Artificial Sequence; identical to SEQ ID NO: 8
  source: /note="Description of Artificial Sequence: Synthetic polypeptide"

SEQ ID NO: 31 - protein, 450 aa, Artificial Sequence
  source: /note="Description of Artificial Sequence: Synthetic polypeptide"
QVQLQESGPGLVKPSETLSLTCTVSGGSISRRNDYWAWIRQSPGKDLEWIGTISFSGSTFYNPSLKSRVTISADTFNNHFSLRLDAVAAADTAVYYCARLSPFVGAAWWFDPWGPGTLVTVSSASTKGPSVFPLAPCSRSTSESTAALGCLVKDYFPEPVTVSWNSGALTSGVHTFPAVLQSSGLYSLSSVVTVPSSSLGTKTYTCNVDHKPSNTKVDKRVESKYGPPCPPCPAPEFLGGPSVFLFPPKPKDTLMISRTPEVTCVVVDVSQEDPEVQFNWYVDGVEVHNAKTKPREEQFNSTYRVVSVLTVLHQDWLNGKEYKCKVSNKGLPSSIEKTISKAKGQPREPQVYTLPPSQEEMTKNQVSLTCLVKGFYPSDIAVEWESNGQPENNYKTTPPVLDSDGSFFLYSRLTVDKSRWQEGNVFSCSVMHEALHNHYTQKSLSLSLGK

SEQ ID NO: 32 - protein, 217 aa, Artificial Sequence; identical to SEQ ID NO: 12
  source: /note="Description of Artificial Sequence: Synthetic polypeptide"

SEQ ID NO: 33 - protein, 454 aa, Artificial Sequence
  source: /note="Description of Artificial Sequence: Synthetic polypeptide"
QLQLQESGPGLVKPSETLSLTCTASGGSITNNIDYWVWIRQPPGRGLEWIGTIYYSGSTFYNPSLKSRVTISVDTSNNQFSLNLNSMSAADTAVYYCARLRYYYDSNGYLPYWIDSWGQGTLVTVSSASTKGPSVFPLAPCSRSTSESTAALGCLVKDYFPEPVTVSWNSGALTSGVHTFPAVLQSSGLYSLSSVVTVPSSSLGTKTYTCNVDHKPSNTKVDKRVESKYGPPCPPCPAPEFLGGPSVFLFPPKPKDTLMISRTPEVTCVVVDVSQEDPEVQFNWYVDGVEVHNAKTKPREEQFNSTYRVVSVLTVLHQDWLNGKEYKCKVSNKGLPSSIEKTISKAKGQPREPQVYTLPPSQEEMTKNQVSLTCLVKGFYPSDIAVEWESNGQPENNYKTTPPVLDSDGSFFLYSRLTVDKSRWQEGNVFSCSVMHEALHNHYTQKSLSLSLGK

SEQ ID NO: 34 - protein, 217 aa, Artificial Sequence; identical to SEQ ID NO: 14
  source: /note="Description of Artificial Sequence: Synthetic polypeptide"

SEQ ID NO: 35 - protein, 452 aa, Artificial Sequence
  source: /note="Description of Artificial Sequence: Synthetic polypeptide"
QLQLQESGPGLVKPSESLSLTCTVSGGSIISNDYYWAWIRQSPGKGLEWIGSINYRGSTFYSPSLNSRVTTSVDTSKNQFFLKLTSVTAADTAMYFCTRLHGRYRGVGRLAFDYWGQGTLVTVSSASTKGPSVFPLAPCSRSTSESTAALGCLVKDYFPEPVTVSWNSGALTSGVHTFPAVLQSSGLYSLSSVVTVPSSSLGTKTYTCNVDHKPSNTKVDKRVESKYGPPCPPCPAPEFLGGPSVFLFPPKPKDTLMISRTPEVTCVVVDVSQEDPEVQFNWYVDGVEVHNAKTKPREEQFNSTYRVVSVLTVLHQDWLNGKEYKCKVSNKGLPSSIEKTISKAKGQPREPQVYTLPPSQEEMTKNQVSLTCLVKGFYPSDIAVEWESNGQPENNYKTTPPVLDSDGSFFLYSRLTVDKSRWQEGNVFSCSVMHEALHNHYTQKSLSLSLGK

SEQ ID NO: 36 - protein, 214 aa, Artificial Sequence; identical to SEQ ID NO: 16
  source: /note="Description of Artificial Sequence: Synthetic polypeptide"

SEQ ID NO: 37 - protein, 453 aa, Artificial Sequence
  source: /note="Description of Artificial Sequence: Synthetic polypeptide"
QVQLQEAGPGLVKPSETLSLTCTVSGGSINTRNYYWGWVRQPPGKGLEWIASVYYTGSTFYDPSLRSRVTISIDTPRNQFSLRVSSVDAGDMGVYYCVRLDGGYNNGYYYYGMDVWGQGTSVTVSSASTKGPSVFPLAPCSRSTSESTAALGCLVKDYFPEPVTVSWNSGALTSGVHTFPAVLQSSGLYSLSSVVTVPSSSLGTKTYTCNVDHKPSNTKVDKRVESKYGPPCPPCPAPEFLGGPSVFLFPPKPKDTLMISRTPEVTCVVVDVSQEDPEVQFNWYVDGVEVHNAKTKPREEQFNSTYRVVSVLTVLHQDWLNGKEYKCKVSNKGLPSSIEKTISKAKGQPREPQVYTLPPSQEEMTKNQVSLTCLVKGFYPSDIAVEWESNGQPENNYKTTPPVLDSDGSFFLYSRLTVDKSRWQEGNVFSCSVMHEALHNHYTQKSLSLSLGK

SEQ ID NO: 38 - protein, 214 aa, Artificial Sequence; identical to SEQ ID NO: 18
  source: /note="Description of Artificial Sequence: Synthetic polypeptide"

SEQ ID NO: 39 - protein, 454 aa, Artificial Sequence
  source: /note="Description of Artificial Sequence: Synthetic polypeptide"
QLQLQESGPGLVKPSETLSLSCAVSGASIRSNTYYWGWIRQPPGRGLEWIGSISHRGDAHYSPSLKSPVTISVDTSKNEFSLKATSVTAADTAVYYCVSLAYSFSWNTYYFYGMDVWGHGITVTVSSASTKGPSVFPLAPCSRSTSESTAALGCLVKDYFPEPVTVSWNSGALTSGVHTFPAVLQSSGLYSLSSVVTVPSSSLGTKTYTCNVDHKPSNTKVDKRVESKYGPPCPPCPAPEFLGGPSVFLFPPKPKDTLMISRTPEVTCVVVDVSQEDPEVQFNWYVDGVEVHNAKTKPREEQFNSTYRVVSVLTVLHQDWLNGKEYKCKVSNKGLPSSIEKTISKAKGQPREPQVYTLPPSQEEMTKNQVSLTCLVKGFYPSDIAVEWESNGQPENNYKTTPPVLDSDGSFFLYSRLTVDKSRWQEGNVFSCSVMHEALHNHYTQKSLSLSLGK

SEQ ID NO: 40 - protein, 217 aa, Artificial Sequence; identical to SEQ ID NO: 20
  source: /note="Description of Artificial Sequence: Synthetic polypeptide"